European Patent Specification EP 3 814 331 B9, published August 9, 2023. Title: Novel LXR modulators with bicyclic core moiety. Applicant: Phenex-FXR GmbH. Application not yet assigned. The sequence listing filed with the application follows.

SEQUENCE LISTING (19 sequences)

SEQ ID NO: 1 - DNA, 1344 bp, Artificial Sequence
  DNA-Sequence LXR alpha-full length
atgtccttgtggctgggggcccctgtgcctgacattcctcctgactctgcggtggagctgtggaagccaggcgcacaggatgcaagcagccaggcccagggaggcagcagctgcatcctcagagaggaagccaggatgccccactctgctgggggtactgcaggggtggggctggaggctgcagagcccacagccctgctcaccagggcagagcccccttcagaacccacagagatccgtccacaaaagcggaaaaaggggccagcccccaaaatgctggggaacgagctatgcagtgtgtgtggggacaaggcctcgggcttccactacaatgttctgagctgcgagggctgcaagggattcttccgccgcagcgtcatcaagggagcgcactacatctgccacagtggcggccactgccccatggacacctacatgcgtcgcaagtgccaggagtgtcggcttcgcaaatgccgtcaggctggcatgcgggaggagtgtgtcctgtcagaagaacagatccgcctgaagaaactgaagcggcaagaggaggaacaggctcatgccacatccttgccccccagggcttcctcacccccccaaatcctgccccagctcagcccggaacaactgggcatgatcgagaagctcgtcgctgcccagcaacagtgtaaccggcgctccttttctgaccggcttcgagtcacgccttggcccatggcaccagatccccatagccgggaggcccgtcagcagcgctttgcccacttcactgagctggccatcgtctctgtgcaggagatagttgactttgctaaacagctacccggcttcctgcagctcagccgggaggaccagattgccctgctgaagacctctgcgatcgaggtgatgcttctggagacatctcggaggtacaaccctgggagtgagagtatcaccttcctcaaggatttcagttataaccgggaagactttgccaaagcagggctgcaagtggaattcatcaaccccatcttcgagttctccagggccatgaatgagctgcaactcaatgatgccgagtttgccttgctcattgctatcagcatcttctctgcagaccggcccaacgtgcaggaccagctccaggtagagaggctgcagcacacatatgtggaagccctgcatgcctacgtctccatccaccatccccatgaccgactgatgttcccacggatgctaatgaaactggtgagcctccggaccctgagcagcgtccactcagagcaagtgtttgcactgcgtctgcaggacaaaaagctcccaccgctgctctctgagatctgggatgtgcacgaatga

SEQ ID NO: 2 - DNA, 1386 bp, Artificial Sequence
  DNA-Sequence LXR beta-full length
atgtcctctcctaccacgagttccctggatacccccctgcctggaaatggcccccctcagcctggcgccccttcttcttcacccactgtaaaggaggagggtccggagccgtggcccgggggtccggaccctgatgtcccaggcactgatgaggccagctcagcctgcagcacagactgggtcatcccagatcccgaagaggaaccagagcgcaagcgaaagaagggcccagccccgaagatgctgggccacgagctttgccgtgtctgtggggacaaggcctccggcttccactacaacgtgctcagctgcgaaggctgcaagggcttcttccggcgcagtgtggtccgtggtggggccaggcgctatgcctgccggggtggcggaacctgccagatggacgctttcatgcggcgcaagtgccagcagtgccggctgcgcaagtgcaaggaggcagggatgagggagcagtgcgtcctttctgaagaacagatccggaagaagaagattcggaaacaacagcagcaggagtcacagtcacagtcgcagtcacctgtggggccgcagggcagcagcagctcagcctctgggcctggggcttcccctggtggatctgaggcaggcagccagggctccggggaaggcgagggcgtccagctaacagcggctcaagaactaatgatccagcagttggtggcggcccaactgcagtgcaacaaacgctccttctccgaccagcccaaagtcacgccctggcccctgggcgcagacccccagtcccgagatgcccgccagcaacgctttgcccacttcacggagctggccatcatctcagtccaggagatcgtggacttcgctaagcaagtgcctggtttcctgcagctgggccgggaggaccagatcgccctcctgaaggcatccactatcgagatcatgctgctagagacagccaggcgctacaaccacgagacagagtgtatcaccttcttgaaggacttcacctacagcaaggacgacttccaccgtgcaggcctgcaggtggagttcatcaaccccatcttcgagttctcgcgggccatgcggcggctgggcctggacgacgctgagtacgccctgctcatcgccatcaacatcttctcggccgaccggcccaacgtgcaggagccgggccgcgtggaggcgttgcagcagccctacgtggaggcgctgctgtcctacacgcgcatcaagaggccgcaggaccagctgcgcttcccgcgcatgctcatgaagctggtgagcctgcgcacgctgagctctgtgcactcggagcaggtcttcgccttgcggctccaggacaagaagctgccgcctctgctgtcggagatctgggacgtccacgagtga

SEQ ID NO: 3 - DNA, 882 bp, Artificial Sequence
  DNA-Sequence LXR alpha-LBD
cttcgcaaatgccgtcaggctggcatgcgggaggagtgtgtcctgtcagaagaacagatccgcctgaagaaactgaagcggcaagaggaggaacaggctcatgccacatccttgccccccagggcttcctcacccccccaaatcctgccccagctcagcccggaacaactgggcatgatcgagaagctcgtcgctgcccagcaacagtgtaaccggcgctccttttctgaccggcttcgagtcacgccttggcccatggcaccagatccccatagccgggaggcccgtcagcagcgctttgcccacttcactgagctggccatcgtctctgtgcaggagatagttgactttgctaaacagctacccggcttcctgcagctcagccgggaggaccagattgccctgctgaagacctctgcgatcgaggtgatgcttctggagacatctcggaggtacaaccctgggagtgagagtatcaccttcctcaaggatttcagttataaccgggaagactttgccaaagcagggctgcaagtggaattcatcaaccccatcttcgagttctccagggccatgaatgagctgcaactcaatgatgccgagtttgccttgctcattgctatcagcatcttctctgcagaccggcccaacgtgcaggaccagctccaggtagagaggctgcagcacacatatgtggaagccctgcatgcctacgtctccatccaccatccccatgaccgactgatgttcccacggatgctaatgaaactggtgagcctccggaccctgagcagcgtccactcagagcaagtgtttgcactgcgtctgcaggacaaaaagctcccaccgctgctctctgagatctgggatgtgcacgaatga

SEQ ID NO: 4 - DNA, 1011 bp, Artificial Sequence
  DNA-sequence LXR beta-LBD
gagcagtgcgtcctttctgaagaacagatccggaagaagaagattcggaaacaacagcagcaggagtcacagtcacagtcgcagtcacctgtggggccgcagggcagcagcagctcagcctctgggcctggggcttcccctggtggatctgaggcaggcagccagggctccggggaaggcgagggtgtccagctaacagcggctcaagaactaatgatccagcagttggtggcggcccaactgcagtgcaacaaacgctccttctccgaccagcccaaagtcacgccctggcccctgggcgcagacccccagtcccgagatgcccgccagcaacgctttgcccacttcacggagctggccatcatctcagtccaggagatcgtggacttcgctaagcaagtgcctggtttcctgcagctgggccgggaggaccagatcgccctcctgaaggcatccactatcgagatcatgctgctagagacagccaggcgctacaaccacgagacagagtgtatcaccttcttgaaggacttcacctacagcaaggacgacttccaccgtgcaggcctgcaggtggagttcatcaaccccatcttcgagttctcgcgggccatgcggcggctgggcctggacgacgctgagtacgccctgctcatcgccatcaacatcttctcggccgaccggcccaacgtgcaggagccgggccgcgtggaggcgttgcagcagccctacgtggaggcgctgctgtcctacacgcgcatcaagaggccgcaggaccagctgcgcttcccgcgcatgctcatgaagctggtgagcctgcgcacgctgagctctgtgcactcggagcaggtcttcgccttgcggctccaggacaagaagctgccgcctctgctgtcggagatctgggacgtccacgagtgaggggctggccacccagccccacagccttgcctgaccaccctccagcagatagacgccggcaccccttcctcttcctctgcttttatttaa

SEQ ID NO: 5 - DNA, 1011 bp, Artificial Sequence
  DNA-sequence SRC1-fragment
gttggcttctctgccagttctccagtcctcaggcagatgagctcacagaattcacctagcagattaaatatacaaccagcaaaagctgagtccaaagataacaaagagattgcctcaattttaaatgaaatgattcaatctgacaacagctctagtgatggcaaacctctggattcagggcttctgcataacaatgacagactttcagatggagacagtaaatactctcaaaccagtcacaaactagtgcagcttttgacaacaactgccgaacagcagttacggcatgctgatatagacacaagctgcaaagatgtcctgtcttgcacaggcacttccaactctgcctctgctaactcttcaggaggttcttgtccctcttctcatagctcattgacagaacggcataaaattctacaccggctcttacaggagggtagcccctcagatatcaccactttgtctgtcgagcctgataaaaaggacagtgcatctacttctgtgtcagtgactggacaggtacaaggaaactccagtataaaactagaactggatgcttcaaagaaaaaagaatcaaaagaccatcagctcctacgctatcttttagataaagatgagaaagatttaagatcaactccaaacctgagcctggatgatgtaaaggtgaaagtggaaaagaaagaacagatggatccatgtaatacaaacccaaccccaatgaccaaacccactcctgaggaaataaaactggaggcccagagccagtttacagctgaccttgaccagtttgatcagttactgcccacgctggagaaggcagcacagttgccaggcttatgtgagacagacaggatggatggtgcggtcaccagtgtaaccatcaaatcggagatcctgccagcttcacttcagtccgccactgccagacccacttccaggctaaatagattacctgagctggaattggaagcaattgataaccaatttggacaaccaggaacaggcgattag

SEQ ID NO: 6 - DNA, 1225 bp, Artificial Sequence
  DNA-sequence NCoR-fragment
gataaagggcctcctccaaaatccagatatgaggaagagctaaggaccagagggaagactaccattactgcagctaacttcatagacgtgatcatcacccggcaaattgcctcggacaaggatgcgagggaacgtggctctcaaagttcagactcttctagtagcttatcttctcacaggtatgaaacacctagcgatgctattgaggtgataagtcctgccagctcacctgcgccaccccaggagaaactgcagacctatcagccagaggttgttaaggcaaatcaagcggaaaatgatcctaccagacaatatgaaggaccattacatcactatcgaccacagcaggaatcaccatctccccaacaacagctgcccccttcttcacaggcagagggaatggggcaagtgcccaggacccatcggctgatcacacttgctgatcacatctgtcaaattatcacacaagattttgctagaaatcaagtttcctcgcagactccccagcagcctcctacttctacattccagaactcaccttctgctttggtatctacacctgtgaggactaaaacatcaaaccgttacagcccagaatcccaggctcagtctgtccatcatcaaagaccaggttcaagggtctctacagaaaatcttgtggacaaatccaggggaagtaggcctggaaaatccccagagaggagtcacgtctcttcggagccctacgagcccatctccccaccccaggttccggttgtgcatgagaaacaggacagcttgctgctcttgtctcagaggggcgcagagcctgcagagcagaggaatgatgcccgctcaccagggagtataagctacttgccttcattcttcaccaagcttgaaaatacatcacccatggttaaatcaaagaagcaggagatttttcgtaagttgaactcctctggtggaggtgactctgatatggcagctgctcagccaggaactgagatctttaatctgccagcagttactacgtcaggctcagttagctctagaggccattcttttgctgatcctgccagtaatcttgggctggaagacattatcaggaaggctctcatgggaagctttgatgacaaagttgaggatcatggagttgtcatgtcccagcctatgggagtagtgcctggtactgccaacacctcagttgtgaccagtggtgagacacgaagagaggaaggggtga

SEQ ID NO: 7 - protein, 25 aa, Artificial Sequence
  Peptide
ENQRGPLESKGHKKLLQLLTCSSDD

SEQ ID NO: 8 - DNA, 20 bp, Artificial Sequence
  Forward primer
cccctctgttaattggctcc

SEQ ID NO: 9 - DNA, 20 bp, Artificial Sequence
  Reverse primer
ttgtggaagtgcaggttagg

SEQ ID NO: 10 - DNA, 22 bp, Artificial Sequence
  Sequence probe
caggctcagggtgtcccatgtt

SEQ ID NO: 11 - DNA, 20 bp, Artificial Sequence
  Forward primer
ctgacctgaaagccgagaag

SEQ ID NO: 12 - DNA, 20 bp, Artificial Sequence
  Reverse primer
agaaggtgctaacgaacagg

SEQ ID NO: 13 - DNA, 25 bp, Artificial Sequence
  Sequence probe
tgtttacaaaagtctcgccccagca

SEQ ID NO: 14 - DNA, 20 bp, Artificial Sequence
  Forward primer
ccatcgactacatccgcttc

SEQ ID NO: 15 - DNA, 20 bp, Artificial Sequence
  Reverse primer
gccctccatagacacatctg

SEQ ID NO: 16 - DNA, 24 bp, Artificial Sequence
  Sequence probe
tctcctgcttgagcttctggttgc

SEQ ID NO: 17 - DNA, 21 bp, Artificial Sequence
  Forward primer
caccaatgactcctatgaccc

SEQ ID NO: 18 - DNA, 23 bp, Artificial Sequence
  Reverse primer
caagtttacagccaagattcacg

SEQ ID NO: 19 - DNA, 20 bp, Artificial Sequence
  Sequence probe
actcctgccacaccagcctc